European Patent Application EP 4 406 547 A1, published July 31, 2024. Title: USE OF POLYPEPTIDE FOR TREATING DEPRESSION OR ANXIETY, AND COMPLEX. Applicant: Shenzhen Chenyang Biological Technology Co., LTD. The sequence listing filed with the application follows.

SEQUENCE LISTING (3 sequences)

SEQ ID NO: 1 - protein, 15 aa, synthetic construct
SKDNSDGVNEKVSCV

SEQ ID NO: 2 - DNA, 45 bp, synthetic construct
  source 1..45: mol_type = other DNA
tctaaagacaatagcgacggagtgaatgaaaaggtgagctgtgtg

SEQ ID NO: 3 - protein, 11 aa, synthetic construct
YGRKKRRQRRR